European Patent Specification EP 3 673 267 B1, published February 25, 2026. Title: METHODS OF DIAGNOSING AND TREATING LUNG CANCER. Applicant: Savicell Diagnostic Ltd. Ramot at Tel-Aviv University Ltd. DAVIDOVITS, Giora PATOLSKY, Fernando DAVIDOVITS, David Eyal ARBEL, Irit TIRMAN, Shoval LUTATY, Aviv SCIENMANN, Tali TIROSH, Reuven PERETZ-SOROKA, Hagit. The sequence listing filed with the application follows.

SEQUENCE LISTING (51 sequences)

SEQ ID NO: 1 - protein, 26 aa, Artificial sequence
  Synthetic peptide
HGRTQDENPVVHFFKNIVTPRTPPPS

SEQ ID NO: 2 - protein, 21 aa, Artificial sequence
  Synthetic peptide
ENPVVHFFKNIVTPRTPPPSQ

SEQ ID NO: 3 - protein, 27 aa, Artificial sequence
  Synthetic peptide
TENPVVHFFKNIVTPRTPPPSQGKGRG

SEQ ID NO: 4 - protein, 13 aa, Artificial sequence
  Synthetic peptide
VHFFKNIVTPRTP

SEQ ID NO: 5 - protein, 26 aa, Artificial sequence
  Synthetic peptide
DENPVVHFFKNIVTPRTPPPSQGKGR

SEQ ID NO: 6 - protein, 21 aa, Artificial sequence
  Synthetic peptide
PPDSSYLSGANLNLSCHSASN

SEQ ID NO: 7 - protein, 9 aa, Artificial sequence
  Synthetic peptide
YLSGANLNL

SEQ ID NO: 8 - protein, 20 aa, Artificial sequence
  Synthetic peptide
IISPPDSSYLSGANLNLSCH

SEQ ID NO: 9 - protein, 29 aa, Artificial sequence
  Synthetic peptide
TPIISPPDSSYLSGANLNLSCHSASNPSP

SEQ ID NO: 10 - protein, 21 aa, Artificial sequence
  Synthetic peptide
PPDSSYSLGANLNLSCHSASN

SEQ ID NO: 11 - protein, 9 aa, Artificial sequence
  Synthetic peptide
YSLGANLNL

SEQ ID NO: 12 - protein, 20 aa, Artificial sequence
  Synthetic peptide
IISPPDSSYSLGANLNLSCH

SEQ ID NO: 13 - protein, 29 aa, Artificial sequence
  Synthetic peptide
TPIISPPDSSYSLGANLNLSCHSASNPSP

SEQ ID NO: 14 - protein, 29 aa, Artificial sequence
  Synthetic peptide
IAKITPNNNGTYACFVSNLATGRNNSIVK

SEQ ID NO: 15 - protein, 21 aa, Artificial sequence
  Synthetic peptide
PNNNGTYACFVSNLATGRNNS

SEQ ID NO: 16 - protein, 20 aa, Artificial sequence
  Synthetic peptide
ITPNNNGTYACFVSNLATGR

SEQ ID NO: 17 - protein, 9 aa, Artificial sequence
  Synthetic peptide
TYACFVSNL

SEQ ID NO: 18 - protein, 20 aa, Artificial sequence
  Synthetic peptide
PDTRPAPGSTAPPAHGVTSA

SEQ ID NO: 19 - protein, 40 aa, Artificial sequence
  Synthetic peptide
APPAHGVTSAPDTRPAPGSTAPPAHGVTSAPDTRPAPGST

SEQ ID NO: 20 - protein, 30 aa, Artificial sequence
  Synthetic peptide
GVTSAPDTRPAPGSTAPPAHGVTSAPDTRP

SEQ ID NO: 21 - protein, 35 aa, Artificial sequence
  Synthetic peptide
AHGVTSAPDTRPAPGSTAPPAHGVTSAPDTRPAPG

SEQ ID NO: 22 - protein, 40 aa, Artificial sequence
  Synthetic peptide
RCGARGPESRLLEFYLAMPFATPMEAELARRSLAQDAPPL

SEQ ID NO: 23 - protein, 26 aa, Artificial sequence
  Synthetic peptide
SRLLEFYLAMPFATPMEAELARRSLA

SEQ ID NO: 24 - protein, 32 aa, Artificial sequence
  Synthetic peptide
GPESRLLEFYLAMPFATPMEAELARRSLAQDA

SEQ ID NO: 25 - protein, 20 aa, Artificial sequence
  Synthetic peptide
LLEFYLAMPFATPMEAELAR

SEQ ID NO: 26 - protein, 19 aa, Artificial sequence
  Synthetic peptide
GSDPACYEFLWGPRALVET

SEQ ID NO: 27 - protein, 9 aa, Artificial sequence
  Synthetic peptide
FLWGPRALV

SEQ ID NO: 28 - protein, 17 aa, Artificial sequence
  Synthetic peptide
EFLWGPRALVETSYVKV

SEQ ID NO: 29 - protein, 29 aa, Artificial sequence
  Synthetic peptide
VPGSDPACYEFLWGPRALVETSYVKVLHH

SEQ ID NO: 30 - protein, 33 aa, Artificial sequence
  Synthetic peptide
RAVPLPAGGGTVLTKMYPRGNHWAVGHLMGKKS

SEQ ID NO: 31 - protein, 36 aa, Artificial sequence
  Synthetic peptide
LAPRGRAVPLPAGGGTVLTKMYPRGNHWAVGHLMGK

SEQ ID NO: 32 - protein, 27 aa, Artificial sequence
  Synthetic peptide
VPLPAGGGTVLTKMYPRGNHWAVGHLM

SEQ ID NO: 33 - protein, 47 aa, Artificial sequence
  Synthetic peptide
VLCLAPRGRAVPLPAGGGTVLTKMYPRGNHWAVGHLMGKKSTGESSS

SEQ ID NO: 34 - protein, 14 aa, Artificial sequence
  Synthetic peptide
MYPRGNHWAVGHLM

SEQ ID NO: 35 - protein, 27 aa, Artificial sequence
  Synthetic peptide
PAGGGTVLTKMYPRGNHWAVGHLMGKK

SEQ ID NO: 36 - protein, 39 aa, Artificial sequence
  Synthetic peptide
RGRAVPLPAGGGTVLTKMYPRGNHWAVGHLMGKKSTGES

SEQ ID NO: 37 - protein, 29 aa, Artificial sequence
  Synthetic peptide
GGTVLTKMYPRGNHWAVGHLMGKKSTGES

SEQ ID NO: 38 - protein, 5 aa, Artificial sequence
  Synthetic peptide
  MISC_FEATURE (1)..(1): 5'   palmitoyl group
KTTKS

SEQ ID NO: 39 - protein, 24 aa, Artificial sequence
  Synthetic peptide
KFPDEEGACQPCPINCTHSCVDLD

SEQ ID NO: 40 - protein, 22 aa, Artificial sequence
  Synthetic peptide
GACQPCPINCTHSCVDLDDKGC

SEQ ID NO: 41 - protein, 30 aa, Artificial sequence
  Synthetic peptide
IWKFPDEEGACQPCPINCTHSCVDLDDKGC

SEQ ID NO: 42 - protein, 10 aa, Artificial sequence
  Synthetic peptide
CQPCPINCTH

SEQ ID NO: 43 - protein, 27 aa, Artificial sequence
  Synthetic peptide
MSWRGRSTYYWPRPRRYVQPPEMIGPM

SEQ ID NO: 44 - protein, 15 aa, Artificial sequence
  Synthetic peptide
STYYWPRPRRYVQPP

SEQ ID NO: 45 - protein, 20 aa, Artificial sequence
  Synthetic peptide
GRSTYYWPRPRRYVQPPEMI

SEQ ID NO: 46 - protein, 9 aa, Artificial sequence
  Synthetic peptide
YYWPRPRRY

SEQ ID NO: 47 - protein, 8 aa, Artificial sequence
  Synthetic peptide
YRPRPRRY

SEQ ID NO: 48 - protein, 29 aa, Artificial sequence
  Synthetic peptide
LVRDKITGQSLGYGFVNYIDPKDAEKAIN

SEQ ID NO: 49 - protein, 16 aa, Artificial sequence
  Synthetic peptide
GQSLGYGFVNYIDPKD

SEQ ID NO: 50 - protein, 9 aa, Artificial sequence
  Synthetic peptide
LGYGFVNYI

SEQ ID NO: 51 - protein, 23 aa, Artificial sequence
  Synthetic peptide
DKITGQSLGYGFVNYIDPKDAEK